European Patent Specification EP 3 506 925 B1, published September 6, 2023. Title: USE OF CGRP RECEPTOR ANTAGONISTS IN NEUROPROTECTION AND NEUROLOGICAL DISORDERS. Applicant: Soares, Christopher J. The sequence listing filed with the application follows.

SEQUENCE LISTING (58 sequences)

SEQ ID NO: 1 - protein, 32 aa, Artificial Sequence
  Synthetic peptide
ACDTAACVLGRLSQELHRLQTYPRTNVGSKAF

SEQ ID NO: 2 - protein, 32 aa, Artificial Sequence
  Synthetic peptide
ACDTASCVLGRLSQELHRLQTYPRTNVGSKAF

SEQ ID NO: 3 - protein, 32 aa, Artificial Sequence
  Synthetic peptide
ACDTAVCVLGRLSQELHRLQTYPRTNVGSKAF

SEQ ID NO: 4 - protein, 32 aa, Artificial Sequence
  Synthetic peptide
ACNTAACVLGRLSQELHRLQTYPRTNVGSKAF

SEQ ID NO: 5 - protein, 32 aa, Artificial Sequence
  Synthetic peptide
ACVLGACVLGRLSQELHRLQTYPRTNVGSKAF

SEQ ID NO: 6 - protein, 32 aa, Artificial Sequence
  Synthetic peptide
ACRFGACVLGRLSQELHRLQTYPRTNVGSKAF

SEQ ID NO: 7 - protein, 32 aa, Artificial Sequence
  Synthetic peptide
ACNLSACVLGRLSQELHRLQTYPRTNVGSKAF

SEQ ID NO: 8 - protein, 32 aa, Artificial Sequence
  Synthetic peptide
CSNTAACVLGRLSQELHRLQTYPRTNVGSKAF

SEQ ID NO: 9 - protein, 32 aa, Artificial Sequence
  Synthetic peptide
ACDTALCVLGRLSQELHRLQTYPRTNVGSKAF

SEQ ID NO: 10 - protein, 32 aa, Artificial Sequence
  Synthetic peptide
ACDTAICVLGRLSQELHRLQTYPRTNVGSKAF

SEQ ID NO: 11 - protein, 32 aa, Artificial Sequence
  Synthetic peptide
ACNLSVCVLGRLSQELHRLQTYPRTNVGSKAF

SEQ ID NO: 12 - protein, 32 aa, Artificial Sequence
  Synthetic peptide
CSNTAVCVLGRLSQELHRLQTYPRTNVGSKAF

SEQ ID NO: 13 - protein, 31 aa, Artificial Sequence
  Synthetic peptide
ACNLSACVLGRLSQELHRLQTYPTNTGSGTP

SEQ ID NO: 14 - protein, 32 aa, Artificial Sequence
  Synthetic peptide
ACVLGACVLGRLSQELHRLQTYPVDPSSPHSY

SEQ ID NO: 15 - protein, 37 aa, Artificial Sequence
  Synthetic peptide
ACDTAACVTHRLAGLLSRSGGVVKNNFVPTNVGSKAF

SEQ ID NO: 16 - protein, 7 aa, Artificial Sequence
  Synthetic peptide
  VARIANT (1)...(1): Xaa = selected from the group consisting Ala, Cys, Gly, Ile, Leu, Met, Phe, Pro, Trp, and Val
  VARIANT (2)...(2): Xaa = selected from the group consisting of Cys, Ser, and Tyr
  VARIANT (3)...(3): Xaa = selected from the group consisting of Arg, Asn, Asp, Cys, Glu, Gln, His, Lys, Ser, Thr, Tyr, and Val
  VARIANT (4)...(4): Xaa = selected from the group consisting of Arg, Asn, Asp, Glu, Gln, His, Leu, Lys, Phe, Ser, Thr, Tyr, and Val
  VARIANT (5)...(5): Xaa = selected from the group consisting of Ala, Gly, Ile, Leu, Met, Phe, Ser, Typ, and Val
  VARIANT (6)...(6): Xaa = selected from the group consisting of Ala, Gly, Ile, Leu, Met, Phe, Ser, Typ, and Val
  VARIANT (7)...(7): Xaa = Cys
XXXXXXX

SEQ ID NO: 17 - protein, 7 aa, Artificial Sequence
  Synthetic peptide
ACDTAAC

SEQ ID NO: 18 - protein, 7 aa, Artificial Sequence
  Synthetic peptide
ACDTASC

SEQ ID NO: 19 - protein, 7 aa, Artificial Sequence
  Synthetic peptide
ACDTAVC

SEQ ID NO: 20 - protein, 7 aa, Artificial Sequence
  Synthetic peptide
ACNTAAC

SEQ ID NO: 21 - protein, 7 aa, Artificial Sequence
  Synthetic peptide
ACVLGAC

SEQ ID NO: 22 - protein, 7 aa, Artificial Sequence
  Synthetic peptide
ACRFGAC

SEQ ID NO: 23 - protein, 7 aa, Artificial Sequence
  Synthetic peptide
ACDLSAC

SEQ ID NO: 24 - protein, 7 aa, Artificial Sequence
  Synthetic peptide
ACNLSAC

SEQ ID NO: 25 - protein, 7 aa, Artificial Sequence
  Synthetic peptide
CSNTAAC

SEQ ID NO: 26 - protein, 7 aa, Artificial Sequence
  Synthetic peptide
ACDTALC

SEQ ID NO: 27 - protein, 7 aa, Artificial Sequence
  Synthetic peptide
ACDTAIC

SEQ ID NO: 28 - protein, 7 aa, Artificial Sequence
  Synthetic peptide
ACDTALC

SEQ ID NO: 29 - protein, 7 aa, Artificial Sequence
  Synthetic peptide
ACDTAIC

SEQ ID NO: 30 - protein, 7 aa, Artificial Sequence
  Synthetic peptide
ACDLSVC

SEQ ID NO: 31 - protein, 7 aa, Artificial Sequence
  Synthetic peptide
ACDLSVC

SEQ ID NO: 32 - protein, 7 aa, Artificial Sequence
  Synthetic peptide
ACNLSVC

SEQ ID NO: 33 - protein, 7 aa, Artificial Sequence
  Synthetic peptide
CSNTAVC

SEQ ID NO: 34 - protein, 19 aa, Artificial Sequence
  Synthetic peptide
VLGRLSQELHRLQTYPRTN

SEQ ID NO: 35 - protein, 19 aa, Artificial Sequence
  Synthetic peptide
VLGKLSQELHKLQTYPRTN

SEQ ID NO: 36 - protein, 19 aa, Artificial Sequence
  Synthetic peptide
VLGKLSQELHKLQTYPRTD

SEQ ID NO: 37 - protein, 19 aa, Artificial Sequence
  Synthetic peptide
VLGKLSQELHKLQTFPRTN

SEQ ID NO: 38 - protein, 19 aa, Artificial Sequence
  Synthetic peptide
VLGKLSQDIHKLQTYPRTN

SEQ ID NO: 39 - protein, 19 aa, Artificial Sequence
  Synthetic peptide
VLGKLSQELHKMQTYPRTD

SEQ ID NO: 40 - protein, 19 aa, Artificial Sequence
  Synthetic peptide
LLGKLSQELHRLQTYTRTD

SEQ ID NO: 41 - protein, 19 aa, Artificial Sequence
  Synthetic peptide
VLGKLSQDLHKLQTFPRTD

SEQ ID NO: 42 - protein, 19 aa, Artificial Sequence
  Synthetic peptide
MLGKLSQDLHKLQTFPRTD

SEQ ID NO: 43 - protein, 19 aa, Artificial Sequence
  Synthetic peptide
VLGKLSQDIHKLQTHPRTD

SEQ ID NO: 44 - protein, 19 aa, Artificial Sequence
  Synthetic peptide
VLGKLSQDIHKLQTHPRTD

SEQ ID NO: 45 - protein, 6 aa, Artificial Sequence
  Synthetic peptide
  VARIANT (1)...(1): Xaa = selected from the group consisting of Ala, Gly, Ile, Leu, Met, Phe, Pro, Trp, and Val
  VARIANT (2)...(2): Xaa = selected from the group consisting of Ala, Gly, Ile, Leu, Met, Phe, Pro, Trp, and Val
  VARIANT (3)...(3): Xaa = selected from the group consisting of Ser and Tyr
  VARIANT (4)...(4): Xaa = selected from the group consisting of Arg, Asn, Asp, Glu, Gln, His, Lys, Ser, Thr, and Tyr
  VARIANT (5)...(5): Xaa = selected from the group consisting of Ala, Gly, Ile, Leu, Met, Phe, Pro, Trp, and Val
  VARIANT (6)...(6): Xaa = selected from the group consisting of Ala, Gly, Ile, Leu, Met, Phe, Pro, Trp, and Val
XXXXXX

SEQ ID NO: 46 - protein, 6 aa, Artificial Sequence
  Synthetic peptide
VGSKAF

SEQ ID NO: 47 - protein, 6 aa, Artificial Sequence
  Synthetic peptide
VGSKAF

SEQ ID NO: 48 - skipped

SEQ ID NO: 49 - protein, 7 aa, Artificial Sequence
  Synthetic peptide
  VARIANT (6)...(6): Xaa = any amino acid residue other than Thr
ACDTAXC

SEQ ID NO: 50 - protein, 16 aa, Artificial Sequence
  Synthetic peptide
EAAAKEAAAKEAAAKA

SEQ ID NO: 51 - protein, 17 aa, Artificial Sequence
  Synthetic peptide
AKAAAEKAAAEKAAAEA

SEQ ID NO: 52 - protein, 16 aa, Artificial Sequence
  Synthetic peptide
AEAAKAEAAKAEAAKA

SEQ ID NO: 53 - protein, 16 aa, Artificial Sequence
  Synthetic peptide
AKAAEAKAAEAKAAEA

SEQ ID NO: 54-56 - skipped (3 entries)

SEQ ID NO: 57 - protein, 32 aa, Artificial Sequence
  Synthetic peptide
ACDLSACVLGRLSQELHRLQTYPRTNVGSKAF

SEQ ID NO: 58 - protein, 32 aa, Artificial Sequence
  Synthetic peptide
ACDLSVCVLGRLSQELHRLQTYPRTNVGSKAF